European Patent Application EP 4 183 795 A1, published May 24, 2023. Title: ANTIBODY MOLECULES AND PEPTIDE DELIVERY SYSTEMS FOR USE IN ALZHEIMER'S DISEASE AND RELATED DISORDERS. Applicant: TECHNOPHAGE, INVESTIGAÇÃO E DESENVOLVIMENTO EM BIOTECNOLOGIA, SA. Application EP. The sequence listing filed with the application follows.

SEQUENCE LISTING (135 sequences)

SEQ ID NO: 1 - protein, 112 aa, unidentified
  REGION 1..112: note = source = /note="Description of Unknown:rabbit immunoglobulin VL domain polypeptide"
  REGION 1..112: note = source = /note="#2"
ELVMTQTPSPVSAAVGGTVSISCQSSKSVYNNNWLSWFQQKPGQPPKLLIYSASTLASGVSSRFKGSGSGTQFTLTISDVQCDDAATYYCQGEFDCSGDCNVFGGGTELEIL

SEQ ID NO: 2 - protein, 112 aa, unidentified
  REGION 1..112: note = source = /note="Description of Unknown:rabbit immunoglobulin VL domain polypeptide"
  REGION 1..112: note = source = /note="#20"
ELDLTQTPSSKSVPVGDTVTINCQASESVYSNNRLAWFQQKPGQPPKLLIYYASTLASGVPSRFKGSGSGTQFTLTISDVVCDDAATYYCAGYKSSTSDGIAFGGGTEVVVK

SEQ ID NO: 3 - protein, 109 aa, unidentified
  REGION 1..109: note = source = /note="Description of Unknown:rabbit immunoglobulin VL domain polypeptide"
  REGION 1..109: note = source = /note="#6in"
ELDLTQTPSSVSEPVGGTVTIKCQASQSINSYLAWYQQKPGQPPKLLIYRTSTLASGVSSRFKGSGSGTEFTLTISDLECADAATYYCQSYYSASSGWAFGGGTEVVVK

SEQ ID NO: 4 - protein, 108 aa, unidentified
  REGION 1..108: note = source = /note="Description of Unknown:rabbit immunoglobulin VL domain polypeptide"
  REGION 1..108: note = source = /note="#27in"
ELVLTQTPSSVSAAVGGTVTINCQASQSVSNRLAWYQQKPGQPPKLLIYGASRLESGVPSRFRGSGSGTEFTLTISGMKAEDAATYYCQSCYYSVGVTFGAGTNVEIK

SEQ ID NO: 5 - protein, 110 aa, unidentified
  REGION 1..110: note = source = /note="Description of Unknown:rabbit immunoglobulin VL domain polypeptide"
  REGION 1..110: note = source = /note="#1"
ELDLTQTPASVEAAVGGTVTINCQASESISNYLNWYQQKPGQPPKRLIYKASTLASGVPSRFSGSGSGTEFTLTISGVECADAATYYCQQSYSYSNVDNTFGGGTEVVVK

SEQ ID NO: 6 - protein, 109 aa, unidentified
  REGION 1..109: note = source = /note="Description of Unknown:rabbit immunoglobulin VL domain polypeptide"
  REGION 1..109: note = source = /note="#3"
ELVLTQTPASVSEPVGGTVTIKCQASQSIGSYLSWYQQKPGQRPKLLIYDASNLASGVPSRFKGSGSGTEFTLTISDLECADAATYYCQCTYYGSSYYTFGGGTEVVVK

SEQ ID NO: 7 - protein, 112 aa, unidentified
  REGION 1..112: note = source = /note="Description of Unknown:rabbit immunoglobulin VL domain polypeptide"
  REGION 1..112: note = source = /note="#4"
ELDLTQTPSSKSVPVGDTVTINCQASDSVYSNNRLAWFQQKPGQPPKLLIYQASKLASGVPSRFSGSGSGTQFTLTISGVQCDDAATYYCQGAYYSSGWSNGFGGGTEVVVK

SEQ ID NO: 8 - protein, 110 aa, unidentified
  REGION 1..110: note = source = /note="Description of Unknown:rabbit immunoglobulin VL domain polypeptide"
  REGION 1..110: note = source = /note="#5"
ELDLTQTPASVEVAVGGTVTIKCQASQSISTYLSWYQQKAGQRPKLLIYGASNLASGVPSRFKGSGSGTQFTLTISGVECADAATYYCQQGYSSSNVDNAFGGGTELEIL

SEQ ID NO: 9 - protein, 112 aa, unidentified
  REGION 1..112: note = source = /note="Description of Unknown:rabbit immunoglobulin VL domain polypeptide"
  REGION 1..112: note = source = /note="#6"
ELDMTQTPSSKSVPVGDTVTINCQASESVYSNNYLAWYQQKPGQPPKLLIYKASTLASGVSSRFSGSGSGTQFTLTISDVVCDDAGTYYCAGFKGTGTDGNAFGGGTELEIL

SEQ ID NO: 10 - protein, 113 aa, unidentified
  REGION 1..113: note = source = /note="Description of Unknown:rabbit immunoglobulin VL domain polypeptide"
  REGION 1..113: note = source = /note="#7"
ELVLTQTPSSKSVPVGDTVTINCQASDSVYSNNFLSWFQQKPGQPPKLLIYSASTLASGVPSRFKGSGSGTQFTLTISDLECADAATYYCQNYRNIGDYGVPFGGGTEVVVKG

SEQ ID NO: 11 - protein, 111 aa, unidentified
  REGION 1..111: note = source = /note="Description of Unknown:rabbit immunoglobulin VL domain polypeptide"
  REGION 1..111: note = source = /note="#8"
ELVMTQTPSSVSEPVGGTVTIKCQASQNIGGYLAWYQQKPGQPPKLLIYDASTLPSGVPSRFSGSGYGTEFTLTISDLECADAATYYCQCTDYGSSYIYNTFGGGTELEIL

SEQ ID NO: 12 - protein, 111 aa, unidentified
  REGION 1..111: note = source = /note="Description of Unknown:rabbit immunoglobulin VL domain polypeptide"
  REGION 1..111: note = source = /note="#9"
ELDLTQTPSPVSAAVGGTVTISCQSSESVYSNNRLAWYQQKPGQPPKLLIYLASSLASGVPSRFKGSGSGTQFTLTIRDLECDDAATYYCLGYRSGSDGDAFGGGTELEIL

SEQ ID NO: 13 - protein, 110 aa, unidentified
  REGION 1..110: note = source = /note="Description of Unknown:rabbit immunoglobulin VL domain polypeptide"
  REGION 1..110: note = source = /note="#10"
ELDLTQTPASVEVAVGGTVTIKCQASESIGNWLAWYQQKPGQPPKLLIYKASTLASGVPSRFKGSGSGTQFTLTISDVQCDDAATYYCAGGYSSSSDKFPFGGGTELEIL

SEQ ID NO: 14 - protein, 110 aa, unidentified
  REGION 1..110: note = source = /note="Description of Unknown:rabbit immunoglobulin VL domain polypeptide"
  REGION 1..110: note = source = /note="#11"
ELDLTQTPASVEVAVGGTVTINCQASQNIYNYLSWYQQKPGQRPKLLIYRASTLASGVSSRFKGSGSGTEYTLTISGVQCADAATYYCQQGYNIGHVENAFGGGTELEIL

SEQ ID NO: 15 - protein, 112 aa, unidentified
  REGION 1..112: note = source = /note="Description of Unknown:rabbit immunoglobulin VL domain polypeptide"
  REGION 1..112: note = source = /note="#14"
ELVMTQTPSPVSAAVGGTVTINCQASQSVYSNNWLSWYQQKPGQPPKLLIYDASKLASGVPSRFSGSGSGTQFTLTISGVQCDDAATYYCLGGYYSSGWYSAFGGGTELEIL

SEQ ID NO: 16 - protein, 109 aa, unidentified
  REGION 1..109: note = source = /note="Description of Unknown:rabbit immunoglobulin VL domain polypeptide"
  REGION 1..109: note = source = /note="#17"
ELVMTQTPASVSEPVGGTVTIKCQASQSISSYLAWYQQKPGQPPKLLIYAASTLASGVPSRFKGSGSGTQFTLTISDLECADAATYYCQSYYDSSSTNAFGGGTEVVVK

SEQ ID NO: 17 - protein, 112 aa, unidentified
  REGION 1..112: note = source = /note="Description of Unknown:rabbit immunoglobulin VL domain polypeptide"
  REGION 1..112: note = source = /note="#19"
ELVMTQTPSPVSAAVGGTVTISCQASQSVYNNKNLAWYQQKPGQPPKLLIYDASKLASGVSSRFKGSGSGTQFTLTISDLECDDAATYYCAGVYNSNNDACAFGGGTEVVVK

SEQ ID NO: 18 - protein, 111 aa, unidentified; identical to SEQ ID NO: 12
  REGION 1..111: note = source = /note="Description of Unknown:rabbit immunoglobulin VL domain polypeptide"
  REGION 1..111: note = source = /note="#26"

SEQ ID NO: 19 - protein, 108 aa, unidentified
  REGION 1..108: note = source = /note="Description of Unknown:rabbit immunoglobulin VL domain polypeptide"
  REGION 1..108: note = source = /note="#29"
ELDLTQTPSSVEAAVGGTVTIKCQASQSISSYLAWYQQKPGQPPKLLIYRASILASGVPSRFKASGSGTQFTLTISDLECADAATYYCQDHYGISDVAFGGGTELEIL

SEQ ID NO: 20 - protein, 112 aa, unidentified; identical to SEQ ID NO: 7
  REGION 1..112: note = source = /note="Description of Unknown:rabbit immunoglobulin VL domain polypeptide"
  REGION 1..112: note = source = /note="#37"

SEQ ID NO: 21 - protein, 110 aa, unidentified
  REGION 1..110: note = source = /note="Description of Unknown:rabbit immunoglobulin VL domain polypeptide"
  REGION 1..110: note = source = /note="#53"
ELVLTQTPASVSEPVGGTVTIKCQASQSVSDYLAWYQQKPGQPPKLLIYRASTLASGVPSRFKGSGSGTQFTLTISDLECADAATYYCQGGYAGSSYGNAFGGGTELEIL

SEQ ID NO: 22 - protein, 10 aa, Dengue virus 2
  REGION 1..10: note = source = /note="#PepH1"
VQQLTKRFSL

SEQ ID NO: 23 - protein, 14 aa, Dengue virus 2
  REGION 1..14: note = source = /note="#PepH2"
KLFMALVAFLRFLT

SEQ ID NO: 24 - protein, 7 aa, Dengue virus 2
  REGION 1..7: note = source = /note="#PepH3 (PEP+)"
AGILKRW

SEQ ID NO: 25 - protein, 23 aa, Dengue virus 2
  REGION 1..23: note = source = /note="#PepH4"
KSKAINVLRGFRKEIGRMLNILN

SEQ ID NO: 26 - protein, 20 aa, Dengue virus 2
  REGION 1..20: note = source = /note="#PepHM'"
LVAFLRFLTIPPTAGILKRW

SEQ ID NO: 27 - protein, 15 aa, Dengue virus 2
  REGION 1..15: note = source = /note="#PepHR'"
KEIGRMLNILNRRRR

SEQ ID NO: 28 - protein, 132 aa, synthetic construct
  REGION 1..132: note = source = /note="Description of Artificial Sequence: Syntheticpolypeptide construct"
  REGION 1..132: note = source = /note="#2-PEP+"
ELVMTQTPSPVSAAVGGTVSISCQSSKSVYNNNWLSWFQQKPGQPPKLLIYSASTLASGVSSRFKGSGSGTQFTLTISDVQCDDAATYYCQGEFDCSGDCNVFGGGTELEILGSGGGGSGGGGSSAGILKRW

SEQ ID NO: 29 - protein, 135 aa, synthetic construct
  REGION 1..135: note = source = /note="Description of Artificial Sequence: Syntheticpolypeptide construct"
  REGION 1..135: note = source = /note="#2-PepH1"
ELVMTQTPSPVSAAVGGTVSISCQSSKSVYNNNWLSWFQQKPGQPPKLLIYSASTLASGVSSRFKGSGSGTQFTLTISDVQCDDAATYYCQGEFDCSGDCNVFGGGTELEILGSGGGGSGGGGSSVQQLTKRFSL

SEQ ID NO: 30 - protein, 139 aa, synthetic construct
  REGION 1..139: note = source = /note="Description of Artificial Sequence: Syntheticpolypeptide construct"
  REGION 1..139: note = source = /note="#2-PepH2"
ELVMTQTPSPVSAAVGGTVSISCQSSKSVYNNNWLSWFQQKPGQPPKLLIYSASTLASGVSSRFKGSGSGTQFTLTISDVQCDDAATYYCQGEFDCSGDCNVFGGGTELEILGSGGGGSGGGGSSKLFMALVAFLRFLT

SEQ ID NO: 31 - protein, 148 aa, synthetic construct
  REGION 1..148: note = source = /note="Description of Artificial Sequence: Syntheticpolypeptide construct"
  REGION 1..148: note = source = /note="#2-PepH4"
ELVMTQTPSPVSAAVGGTVSISCQSSKSVYNNNWLSWFQQKPGQPPKLLIYSASTLASGVSSRFKGSGSGTQFTLTISDVQCDDAATYYCQGEFDCSGDCNVFGGGTELEILGSGGGGSGGGGSSKSKAINVLRGFRKEIGRMLNILN

SEQ ID NO: 32 - protein, 132 aa, synthetic construct
  REGION 1..132: note = source = /note="Description of Artificial Sequence: Syntheticpolypeptide construct"
  REGION 1..132: note = source = /note="#20-PEP+"
ELDLTQTPSSKSVPVGDTVTINCQASESVYSNNRLAWFQQKPGQPPKLLIYYASTLASGVPSRFKGSGSGTQFTLTISDVVCDDAATYYCAGYKSSTSDGIAFGGGTEVVVKGSGGGGSGGGGSSAGILKRW

SEQ ID NO: 33 - protein, 135 aa, synthetic construct
  REGION 1..135: note = source = /note="Description of Artificial Sequence: Syntheticpolypeptide construct"
  REGION 1..135: note = source = /note="#20-PepH1"
ELDLTQTPSSKSVPVGDTVTINCQASESVYSNNRLAWFQQKPGQPPKLLIYYASTLASGVPSRFKGSGSGTQFTLTISDVVCDDAATYYCAGYKSSTSDGIAFGGGTEVVVKGSGGGGSGGGGSSVQQLTKRFSL

SEQ ID NO: 34 - protein, 139 aa, synthetic construct
  REGION 1..139: note = source = /note="Description of Artificial Sequence: Syntheticpolypeptide construct"
  REGION 1..139: note = source = /note="#20-PepH2"
ELDLTQTPSSKSVPVGDTVTINCQASESVYSNNRLAWFQQKPGQPPKLLIYYASTLASGVPSRFKGSGSGTQFTLTISDVVCDDAATYYCAGYKSSTSDGIAFGGGTEVVVKGSGGGGSGGGGSSKLFMALVAFLRFLT

SEQ ID NO: 35 - protein, 148 aa, synthetic construct
  REGION 1..148: note = source = /note="Description of Artificial Sequence: Syntheticpolypeptide construct"
  REGION 1..148: note = source = /note="#20-PepH4"
ELDLTQTPSSKSVPVGDTVTINCQASESVYSNNRLAWFQQKPGQPPKLLIYYASTLASGVPSRFKGSGSGTQFTLTISDVVCDDAATYYCAGYKSSTSDGIAFGGGTEVVVKGSGGGGSGGGGSSKSKAINVLRGFRKEIGRMLNILN

SEQ ID NO: 36 - protein, 128 aa, synthetic construct
  REGION 1..128: note = source = /note="Description of Artificial Sequence: Syntheticpolypeptide construct"
  REGION 1..128: note = source = /note="#6in-PEP+"
ELDLTQTPSSVSEPVGGTVTIKCQASQSINSYLAWYQQKPGQPPKLLIYRTSTLASGVSSRFKGSGSGTEFTLTISDLECADAATYYCQSYYSASSGWAFGGGTEVVVKSGGGGSGGGGSSAGILKRW

SEQ ID NO: 37 - protein, 131 aa, synthetic construct
  REGION 1..131: note = source = /note="Description of Artificial Sequence: Syntheticpolypeptide construct"
  REGION 1..131: note = source = /note="#6in-PepH1"
ELDLTQTPSSVSEPVGGTVTIKCQASQSINSYLAWYQQKPGQPPKLLIYRTSTLASGVSSRFKGSGSGTEFTLTISDLECADAATYYCQSYYSASSGWAFGGGTEVVVKSGGGGSGGGGSSVQQLTKRFSL

SEQ ID NO: 38 - protein, 135 aa, synthetic construct
  REGION 1..135: note = source = /note="Description of Artificial Sequence: Syntheticpolypeptide construct"
  REGION 1..135: note = source = /note="#6in-PepH2"
ELDLTQTPSSVSEPVGGTVTIKCQASQSINSYLAWYQQKPGQPPKLLIYRTSTLASGVSSRFKGSGSGTEFTLTISDLECADAATYYCQSYYSASSGWAFGGGTEVVVKSGGGGSGGGGSSKLFMALVAFLRFLT

SEQ ID NO: 39 - protein, 144 aa, synthetic construct
  REGION 1..144: note = source = /note="Description of Artificial Sequence: Syntheticpolypeptide construct"
  REGION 1..144: note = source = /note="#6in-PepH4"
ELDLTQTPSSVSEPVGGTVTIKCQASQSINSYLAWYQQKPGQPPKLLIYRTSTLASGVSSRFKGSGSGTEFTLTISDLECADAATYYCQSYYSASSGWAFGGGTEVVVKSGGGGSGGGGSSKSKAINVLRGFRKEIGRMLNILN

SEQ ID NO: 40 - protein, 127 aa, synthetic construct
  REGION 1..127: note = source = /note="Description of Artificial Sequence: Syntheticpolypeptide construct"
  REGION 1..127: note = source = /note="#27in-PEP+"
ELVLTQTPSSVSAAVGGTVTINCQASQSVSNRLAWYQQKPGQPPKLLIYGASRLESGVPSRFRGSGSGTEFTLTISGMKAEDAATYYCQSCYYSVGVTFGAGTNVEIKSGGGGSGGGGSSAGILKRW

SEQ ID NO: 41 - protein, 130 aa, synthetic construct
  REGION 1..130: note = source = /note="Description of Artificial Sequence: Syntheticpolypeptide construct"
  REGION 1..130: note = source = /note="#27in-PepH1"
ELVLTQTPSSVSAAVGGTVTINCQASQSVSNRLAWYQQKPGQPPKLLIYGASRLESGVPSRFRGSGSGTEFTLTISGMKAEDAATYYCQSCYYSVGVTFGAGTNVEIKSGGGGSGGGGSSVQQLTKRFSL

SEQ ID NO: 42 - protein, 134 aa, synthetic construct
  REGION 1..134: note = source = /note="Description of Artificial Sequence: Syntheticpolypeptide construct"
  REGION 1..134: note = source = /note="#27in-PepH2"
ELVLTQTPSSVSAAVGGTVTINCQASQSVSNRLAWYQQKPGQPPKLLIYGASRLESGVPSRFRGSGSGTEFTLTISGMKAEDAATYYCQSCYYSVGVTFGAGTNVEIKSGGGGSGGGGSSKLFMALVAFLRFLT

SEQ ID NO: 43 - protein, 143 aa, synthetic construct
  REGION 1..143: note = source = /note="Description of Artificial Sequence: Syntheticpolypeptide construct"
  REGION 1..143: note = source = /note="#27in-PepH4"
ELVLTQTPSSVSAAVGGTVTINCQASQSVSNRLAWYQQKPGQPPKLLIYGASRLESGVPSRFRGSGSGTEFTLTISGMKAEDAATYYCQSCYYSVGVTFGAGTNVEIKSGGGGSGGGGSSKSKAINVLRGFRKEIGRMLNILN

SEQ ID NO: 44 - protein, 129 aa, synthetic construct
  REGION 1..129: note = source = /note="Description of Artificial Sequence: Syntheticpolypeptide construct"
  REGION 1..129: note = source = /note="#1-PEP+"
ELDLTQTPASVEAAVGGTVTINCQASESISNYLNWYQQKPGQPPKRLIYKASTLASGVPSRFSGSGSGTEFTLTISGVECADAATYYCQQSYSYSNVDNTFGGGTEVVVKSGGGGSGGGGSSAGILKRW

SEQ ID NO: 45 - protein, 132 aa, synthetic construct
  REGION 1..132: note = source = /note="Description of Artificial Sequence: Syntheticpolypeptide construct"
  REGION 1..132: note = source = /note="#1-PepH1"
ELDLTQTPASVEAAVGGTVTINCQASESISNYLNWYQQKPGQPPKRLIYKASTLASGVPSRFSGSGSGTEFTLTISGVECADAATYYCQQSYSYSNVDNTFGGGTEVVVKSGGGGSGGGGSSVQQLTKRFSL

SEQ ID NO: 46 - protein, 136 aa, synthetic construct
  REGION 1..136: note = source = /note="Description of Artificial Sequence: Syntheticpolypeptide construct"
  REGION 1..136: note = source = /note="#1-PepH2"
ELDLTQTPASVEAAVGGTVTINCQASESISNYLNWYQQKPGQPPKRLIYKASTLASGVPSRFSGSGSGTEFTLTISGVECADAATYYCQQSYSYSNVDNTFGGGTEVVVKSGGGGSGGGGSSKLFMALVAFLRFLT

SEQ ID NO: 47 - protein, 145 aa, synthetic construct
  REGION 1..145: note = source = /note="Description of Artificial Sequence: Syntheticpolypeptide construct"
  REGION 1..145: note = source = /note="#1-PepH4"
ELDLTQTPASVEAAVGGTVTINCQASESISNYLNWYQQKPGQPPKRLIYKASTLASGVPSRFSGSGSGTEFTLTISGVECADAATYYCQQSYSYSNVDNTFGGGTEVVVKSGGGGSGGGGSSKSKAINVLRGFRKEIGRMLNILN

SEQ ID NO: 48 - protein, 128 aa, synthetic construct
  REGION 1..128: note = source = /note="Description of Artificial Sequence: Syntheticpolypeptide construct"
  REGION 1..128: note = source = /note="#3-PEP+"
ELVLTQTPASVSEPVGGTVTIKCQASQSIGSYLSWYQQKPGQRPKLLIYDASNLASGVPSRFKGSGSGTEFTLTISDLECADAATYYCQCTYYGSSYYTFGGGTEVVVKSGGGGSGGGGSSAGILKRW

SEQ ID NO: 49 - protein, 131 aa, synthetic construct
  REGION 1..131: note = source = /note="Description of Artificial Sequence: Syntheticpolypeptide construct"
  REGION 1..131: note = source = /note="#3-PepH1"
ELVLTQTPASVSEPVGGTVTIKCQASQSIGSYLSWYQQKPGQRPKLLIYDASNLASGVPSRFKGSGSGTEFTLTISDLECADAATYYCQCTYYGSSYYTFGGGTEVVVKSGGGGSGGGGSSVQQLTKRFSL

SEQ ID NO: 50 - protein, 135 aa, synthetic construct
  REGION 1..135: note = source = /note="Description of Artificial Sequence: Syntheticpolypeptide construct"
  REGION 1..135: note = source = /note="#3-PepH2"
ELVLTQTPASVSEPVGGTVTIKCQASQSIGSYLSWYQQKPGQRPKLLIYDASNLASGVPSRFKGSGSGTEFTLTISDLECADAATYYCQCTYYGSSYYTFGGGTEVVVKSGGGGSGGGGSSKLFMALVAFLRFLT

SEQ ID NO: 51 - protein, 144 aa, synthetic construct
  REGION 1..144: note = source = /note="Description of Artificial Sequence: Syntheticpolypeptide construct"
  REGION 1..144: note = source = /note="#3-PepH4"
ELVLTQTPASVSEPVGGTVTIKCQASQSIGSYLSWYQQKPGQRPKLLIYDASNLASGVPSRFKGSGSGTEFTLTISDLECADAATYYCQCTYYGSSYYTFGGGTEVVVKSGGGGSGGGGSSKSKAINVLRGFRKEIGRMLNILN

SEQ ID NO: 52 - protein, 131 aa, synthetic construct
  REGION 1..131: note = source = /note="Description of Artificial Sequence: Syntheticpolypeptide construct"
  REGION 1..131: note = source = /note="#4-PEP+"
ELDLTQTPSSKSVPVGDTVTINCQASDSVYSNNRLAWFQQKPGQPPKLLIYQASKLASGVPSRFSGSGSGTQFTLTISGVQCDDAATYYCQGAYYSSGWSNGFGGGTEVVVKSGGGGSGGGGSSAGILKRW

SEQ ID NO: 53 - protein, 134 aa, synthetic construct
  REGION 1..134: note = source = /note="Description of Artificial Sequence: Syntheticpolypeptide construct"
  REGION 1..134: note = source = /note="#4-PepH1"
ELDLTQTPSSKSVPVGDTVTINCQASDSVYSNNRLAWFQQKPGQPPKLLIYQASKLASGVPSRFSGSGSGTQFTLTISGVQCDDAATYYCQGAYYSSGWSNGFGGGTEVVVKSGGGGSGGGGSSVQQLTKRFSL

SEQ ID NO: 54 - protein, 138 aa, synthetic construct
  REGION 1..138: note = source = /note="Description of Artificial Sequence: Syntheticpolypeptide construct"
  REGION 1..138: note = source = /note="#4-PepH2"
ELDLTQTPSSKSVPVGDTVTINCQASDSVYSNNRLAWFQQKPGQPPKLLIYQASKLASGVPSRFSGSGSGTQFTLTISGVQCDDAATYYCQGAYYSSGWSNGFGGGTEVVVKSGGGGSGGGGSSKLFMALVAFLRFLT

SEQ ID NO: 55 - protein, 147 aa, synthetic construct
  REGION 1..147: note = source = /note="Description of Artificial Sequence: Syntheticpolypeptide construct"
  REGION 1..147: note = source = /note="#4-PepH4"
ELDLTQTPSSKSVPVGDTVTINCQASDSVYSNNRLAWFQQKPGQPPKLLIYQASKLASGVPSRFSGSGSGTQFTLTISGVQCDDAATYYCQGAYYSSGWSNGFGGGTEVVVKSGGGGSGGGGSSKSKAINVLRGFRKEIGRMLNILN

SEQ ID NO: 56 - protein, 129 aa, synthetic construct
  REGION 1..129: note = source = /note="Description of Artificial Sequence: Syntheticpolypeptide construct"
  REGION 1..129: note = source = /note="#5-PEP+"
ELDLTQTPASVEVAVGGTVTIKCQASQSISTYLSWYQQKAGQRPKLLIYGASNLASGVPSRFKGSGSGTQFTLTISGVECADAATYYCQQGYSSSNVDNAFGGGTELEILSGGGGSGGGGSSAGILKRW

SEQ ID NO: 57 - protein, 132 aa, synthetic construct
  REGION 1..132: note = source = /note="Description of Artificial Sequence: Syntheticpolypeptide construct"
  REGION 1..132: note = source = /note="#5-PepH1"
ELDLTQTPASVEVAVGGTVTIKCQASQSISTYLSWYQQKAGQRPKLLIYGASNLASGVPSRFKGSGSGTQFTLTISGVECADAATYYCQQGYSSSNVDNAFGGGTELEILSGGGGSGGGGSSVQQLTKRFSL

SEQ ID NO: 58 - protein, 136 aa, synthetic construct
  REGION 1..136: note = source = /note="Description of Artificial Sequence: Syntheticpolypeptide construct"
  REGION 1..136: note = source = /note="#5-PepH2"
ELDLTQTPASVEVAVGGTVTIKCQASQSISTYLSWYQQKAGQRPKLLIYGASNLASGVPSRFKGSGSGTQFTLTISGVECADAATYYCQQGYSSSNVDNAFGGGTELEILSGGGGSGGGGSSKLFMALVAFLRFLT

SEQ ID NO: 59 - protein, 145 aa, synthetic construct
  REGION 1..145: note = source = /note="Description of Artificial Sequence: Syntheticpolypeptide construct"
  REGION 1..145: note = source = /note="#5-PepH4"
ELDLTQTPASVEVAVGGTVTIKCQASQSISTYLSWYQQKAGQRPKLLIYGASNLASGVPSRFKGSGSGTQFTLTISGVECADAATYYCQQGYSSSNVDNAFGGGTELEILSGGGGSGGGGSSKSKAINVLRGFRKEIGRMLNILN

SEQ ID NO: 60 - protein, 131 aa, synthetic construct
  REGION 1..131: note = source = /note="Description of Artificial Sequence: Syntheticpolypeptide construct"
  REGION 1..131: note = source = /note="#6-PEP+"
ELDMTQTPSSKSVPVGDTVTINCQASESVYSNNYLAWYQQKPGQPPKLLIYKASTLASGVSSRFSGSGSGTQFTLTISDVVCDDAGTYYCAGFKGTGTDGNAFGGGTELEILSGGGGSGGGGSSAGILKRW

SEQ ID NO: 61 - protein, 134 aa, synthetic construct
  REGION 1..134: note = source = /note="Description of Artificial Sequence: Syntheticpolypeptide construct"
  REGION 1..134: note = source = /note="#6-PepH1"
ELDMTQTPSSKSVPVGDTVTINCQASESVYSNNYLAWYQQKPGQPPKLLIYKASTLASGVSSRFSGSGSGTQFTLTISDVVCDDAGTYYCAGFKGTGTDGNAFGGGTELEILSGGGGSGGGGSSVQQLTKRFSL

SEQ ID NO: 62 - protein, 138 aa, synthetic construct
  REGION 1..138: note = source = /note="Description of Artificial Sequence: Syntheticpolypeptide construct"
  REGION 1..138: note = source = /note="#6-PepH2"
ELDMTQTPSSKSVPVGDTVTINCQASESVYSNNYLAWYQQKPGQPPKLLIYKASTLASGVSSRFSGSGSGTQFTLTISDVVCDDAGTYYCAGFKGTGTDGNAFGGGTELEILSGGGGSGGGGSSKLFMALVAFLRFLT

SEQ ID NO: 63 - protein, 147 aa, synthetic construct
  REGION 1..147: note = source = /note="Description of Artificial Sequence: Syntheticpolypeptide construct"
  REGION 1..147: note = source = /note="#6-PepH4"
ELDMTQTPSSKSVPVGDTVTINCQASESVYSNNYLAWYQQKPGQPPKLLIYKASTLASGVSSRFSGSGSGTQFTLTISDVVCDDAGTYYCAGFKGTGTDGNAFGGGTELEILSGGGGSGGGGSSKSKAINVLRGFRKEIGRMLNILN

SEQ ID NO: 64 - protein, 132 aa, synthetic construct
  REGION 1..132: note = source = /note="Description of Artificial Sequence: Syntheticpolypeptide construct"
  REGION 1..132: note = source = /note="#7-PEP+"
ELVLTQTPSSKSVPVGDTVTINCQASDSVYSNNFLSWFQQKPGQPPKLLIYSASTLASGVPSRFKGSGSGTQFTLTISDLECADAATYYCQNYRNIGDYGVPFGGGTEVVVKGSGGGGSGGGGSSAGILKRW

SEQ ID NO: 65 - protein, 135 aa, synthetic construct
  REGION 1..135: note = source = /note="Description of Artificial Sequence: Syntheticpolypeptide construct"
  REGION 1..135: note = source = /note="#7-PepH1"
ELVLTQTPSSKSVPVGDTVTINCQASDSVYSNNFLSWFQQKPGQPPKLLIYSASTLASGVPSRFKGSGSGTQFTLTISDLECADAATYYCQNYRNIGDYGVPFGGGTEVVVKGSGGGGSGGGGSSVQQLTKRFSL

SEQ ID NO: 66 - protein, 139 aa, synthetic construct
  REGION 1..139: note = source = /note="Description of Artificial Sequence: Syntheticpolypeptide construct"
  REGION 1..139: note = source = /note="#7-PepH2"
ELVLTQTPSSKSVPVGDTVTINCQASDSVYSNNFLSWFQQKPGQPPKLLIYSASTLASGVPSRFKGSGSGTQFTLTISDLECADAATYYCQNYRNIGDYGVPFGGGTEVVVKGSGGGGSGGGGSSKLFMALVAFLRFLT

SEQ ID NO: 67 - protein, 148 aa, synthetic construct
  REGION 1..148: note = source = /note="Description of Artificial Sequence: Syntheticpolypeptide construct"
  REGION 1..148: note = source = /note="#7-PepH4"
ELVLTQTPSSKSVPVGDTVTINCQASDSVYSNNFLSWFQQKPGQPPKLLIYSASTLASGVPSRFKGSGSGTQFTLTISDLECADAATYYCQNYRNIGDYGVPFGGGTEVVVKGSGGGGSGGGGSSKSKAINVLRGFRKEIGRMLNILN

SEQ ID NO: 68 - protein, 130 aa, synthetic construct
  REGION 1..130: note = source = /note="Description of Artificial Sequence: Syntheticpolypeptide construct"
  REGION 1..130: note = source = /note="#8-PEP+"
ELVMTQTPSSVSEPVGGTVTIKCQASQNIGGYLAWYQQKPGQPPKLLIYDASTLPSGVPSRFSGSGYGTEFTLTISDLECADAATYYCQCTDYGSSYIYNTFGGGTELEILSGGGGSGGGGSSAGILKRW

SEQ ID NO: 69 - protein, 133 aa, synthetic construct
  REGION 1..133: note = source = /note="Description of Artificial Sequence: Syntheticpolypeptide construct"
  REGION 1..133: note = source = /note="#8-PepH1"
ELVMTQTPSSVSEPVGGTVTIKCQASQNIGGYLAWYQQKPGQPPKLLIYDASTLPSGVPSRFSGSGYGTEFTLTISDLECADAATYYCQCTDYGSSYIYNTFGGGTELEILSGGGGSGGGGSSVQQLTKRFSL

SEQ ID NO: 70 - protein, 137 aa, synthetic construct
  REGION 1..137: note = source = /note="Description of Artificial Sequence: Syntheticpolypeptide construct"
  REGION 1..137: note = source = /note="#8-PepH2"
ELVMTQTPSSVSEPVGGTVTIKCQASQNIGGYLAWYQQKPGQPPKLLIYDASTLPSGVPSRFSGSGYGTEFTLTISDLECADAATYYCQCTDYGSSYIYNTFGGGTELEILSGGGGSGGGGSSKLFMALVAFLRFLT

SEQ ID NO: 71 - protein, 146 aa, synthetic construct
  REGION 1..146: note = source = /note="Description of Artificial Sequence: Syntheticpolypeptide construct"
  REGION 1..146: note = source = /note="#8-PepH4"
ELVMTQTPSSVSEPVGGTVTIKCQASQNIGGYLAWYQQKPGQPPKLLIYDASTLPSGVPSRFSGSGYGTEFTLTISDLECADAATYYCQCTDYGSSYIYNTFGGGTELEILSGGGGSGGGGSSKSKAINVLRGFRKEIGRMLNILN

SEQ ID NO: 72 - protein, 130 aa, synthetic construct
  REGION 1..130: note = source = /note="Description of Artificial Sequence: Syntheticpolypeptide construct"
  REGION 1..130: note = source = /note="#9-PEP+"
ELDLTQTPSPVSAAVGGTVTISCQSSESVYSNNRLAWYQQKPGQPPKLLIYLASSLASGVPSRFKGSGSGTQFTLTIRDLECDDAATYYCLGYRSGSDGDAFGGGTELEILSGGGGSGGGGSSAGILKRW

SEQ ID NO: 73 - protein, 133 aa, synthetic construct
  REGION 1..133: note = source = /note="Description of Artificial Sequence: Syntheticpolypeptide construct"
  REGION 1..133: note = source = /note="#9-PepH1"
ELDLTQTPSPVSAAVGGTVTISCQSSESVYSNNRLAWYQQKPGQPPKLLIYLASSLASGVPSRFKGSGSGTQFTLTIRDLECDDAATYYCLGYRSGSDGDAFGGGTELEILSGGGGSGGGGSSVQQLTKRFSL

SEQ ID NO: 74 - protein, 137 aa, synthetic construct
  REGION 1..137: note = source = /note="Description of Artificial Sequence: Syntheticpolypeptide construct"
  REGION 1..137: note = source = /note="#9-PepH2"
ELDLTQTPSPVSAAVGGTVTISCQSSESVYSNNRLAWYQQKPGQPPKLLIYLASSLASGVPSRFKGSGSGTQFTLTIRDLECDDAATYYCLGYRSGSDGDAFGGGTELEILSGGGGSGGGGSSKLFMALVAFLRFLT

SEQ ID NO: 75 - protein, 146 aa, synthetic construct
  REGION 1..146: note = source = /note="Description of Artificial Sequence: Syntheticpolypeptide construct"
  REGION 1..146: note = source = /note="#9-PepH4"
ELDLTQTPSPVSAAVGGTVTISCQSSESVYSNNRLAWYQQKPGQPPKLLIYLASSLASGVPSRFKGSGSGTQFTLTIRDLECDDAATYYCLGYRSGSDGDAFGGGTELEILSGGGGSGGGGSSKSKAINVLRGFRKEIGRMLNILN

SEQ ID NO: 76 - protein, 129 aa, synthetic construct
  REGION 1..129: note = source = /note="Description of Artificial Sequence: Syntheticpolypeptide construct"
  REGION 1..129: note = source = /note="#10-PEP+"
ELDLTQTPASVEVAVGGTVTIKCQASESIGNWLAWYQQKPGQPPKLLIYKASTLASGVPSRFKGSGSGTQFTLTISDVQCDDAATYYCAGGYSSSSDKFPFGGGTELEILSGGGGSGGGGSSAGILKRW

SEQ ID NO: 77 - protein, 132 aa, synthetic construct
  REGION 1..132: note = source = /note="Description of Artificial Sequence: Syntheticpolypeptide construct"
  REGION 1..132: note = source = /note="#10-PepH1"
ELDLTQTPASVEVAVGGTVTIKCQASESIGNWLAWYQQKPGQPPKLLIYKASTLASGVPSRFKGSGSGTQFTLTISDVQCDDAATYYCAGGYSSSSDKFPFGGGTELEILSGGGGSGGGGSSVQQLTKRFSL

SEQ ID NO: 78 - protein, 136 aa, synthetic construct
  REGION 1..136: note = source = /note="Description of Artificial Sequence: Syntheticpolypeptide construct"
  REGION 1..136: note = source = /note="#10-PepH2"
ELDLTQTPASVEVAVGGTVTIKCQASESIGNWLAWYQQKPGQPPKLLIYKASTLASGVPSRFKGSGSGTQFTLTISDVQCDDAATYYCAGGYSSSSDKFPFGGGTELEILSGGGGSGGGGSSKLFMALVAFLRFLT

SEQ ID NO: 79 - protein, 145 aa, synthetic construct
  REGION 1..145: note = source = /note="Description of Artificial Sequence: Syntheticpolypeptide construct"
  REGION 1..145: note = source = /note="#10-PepH4"
ELDLTQTPASVEVAVGGTVTIKCQASESIGNWLAWYQQKPGQPPKLLIYKASTLASGVPSRFKGSGSGTQFTLTISDVQCDDAATYYCAGGYSSSSDKFPFGGGTELEILSGGGGSGGGGSSKSKAINVLRGFRKEIGRMLNILN

SEQ ID NO: 80 - protein, 129 aa, synthetic construct
  REGION 1..129: note = source = /note="Description of Artificial Sequence: Syntheticpolypeptide construct"
  REGION 1..129: note = source = /note="#11-PEP+"
ELDLTQTPASVEVAVGGTVTINCQASQNIYNYLSWYQQKPGQRPKLLIYRASTLASGVSSRFKGSGSGTEYTLTISGVQCADAATYYCQQGYNIGHVENAFGGGTELEILSGGGGSGGGGSSAGILKRW

SEQ ID NO: 81 - protein, 132 aa, synthetic construct
  REGION 1..132: note = source = /note="Description of Artificial Sequence: Syntheticpolypeptide construct"
  REGION 1..132: note = source = /note="#11-PepH1"
ELDLTQTPASVEVAVGGTVTINCQASQNIYNYLSWYQQKPGQRPKLLIYRASTLASGVSSRFKGSGSGTEYTLTISGVQCADAATYYCQQGYNIGHVENAFGGGTELEILSGGGGSGGGGSSVQQLTKRFSL

SEQ ID NO: 82 - protein, 136 aa, synthetic construct
  REGION 1..136: note = source = /note="Description of Artificial Sequence: Syntheticpolypeptide construct"
  REGION 1..136: note = source = /note="#11-PepH2"
ELDLTQTPASVEVAVGGTVTINCQASQNIYNYLSWYQQKPGQRPKLLIYRASTLASGVSSRFKGSGSGTEYTLTISGVQCADAATYYCQQGYNIGHVENAFGGGTELEILSGGGGSGGGGSSKLFMALVAFLRFLT

SEQ ID NO: 83 - protein, 145 aa, synthetic construct
  REGION 1..145: note = source = /note="Description of Artificial Sequence: Syntheticpolypeptide construct"
  REGION 1..145: note = source = /note="#11-PepH4"
ELDLTQTPASVEVAVGGTVTINCQASQNIYNYLSWYQQKPGQRPKLLIYRASTLASGVSSRFKGSGSGTEYTLTISGVQCADAATYYCQQGYNIGHVENAFGGGTELEILSGGGGSGGGGSSKSKAINVLRGFRKEIGRMLNILN

SEQ ID NO: 84 - protein, 131 aa, synthetic construct
  REGION 1..131: note = source = /note="Description of Artificial Sequence: Syntheticpolypeptide construct"
  REGION 1..131: note = source = /note="#14-PEP+"
ELVMTQTPSPVSAAVGGTVTINCQASQSVYSNNWLSWYQQKPGQPPKLLIYDASKLASGVPSRFSGSGSGTQFTLTISGVQCDDAATYYCLGGYYSSGWYSAFGGGTELEILSGGGGSGGGGSSAGILKRW

SEQ ID NO: 85 - protein, 134 aa, synthetic construct
  REGION 1..134: note = source = /note="Description of Artificial Sequence: Syntheticpolypeptide construct"
  REGION 1..134: note = source = /note="#14-PepH1"
ELVMTQTPSPVSAAVGGTVTINCQASQSVYSNNWLSWYQQKPGQPPKLLIYDASKLASGVPSRFSGSGSGTQFTLTISGVQCDDAATYYCLGGYYSSGWYSAFGGGTELEILSGGGGSGGGGSSVQQLTKRFSL

SEQ ID NO: 86 - protein, 138 aa, synthetic construct
  REGION 1..138: note = source = /note="Description of Artificial Sequence: Syntheticpolypeptide construct"
  REGION 1..138: note = source = /note="#14-PepH2"
ELVMTQTPSPVSAAVGGTVTINCQASQSVYSNNWLSWYQQKPGQPPKLLIYDASKLASGVPSRFSGSGSGTQFTLTISGVQCDDAATYYCLGGYYSSGWYSAFGGGTELEILSGGGGSGGGGSSKLFMALVAFLRFLT

SEQ ID NO: 87 - protein, 147 aa, synthetic construct
  REGION 1..147: note = source = /note="Description of Artificial Sequence: Syntheticpolypeptide construct"
  REGION 1..147: note = source = /note="#14-PepH4"
ELVMTQTPSPVSAAVGGTVTINCQASQSVYSNNWLSWYQQKPGQPPKLLIYDASKLASGVPSRFSGSGSGTQFTLTISGVQCDDAATYYCLGGYYSSGWYSAFGGGTELEILSGGGGSGGGGSSKSKAINVLRGFRKEIGRMLNILN

SEQ ID NO: 88 - protein, 128 aa, synthetic construct
  REGION 1..128: note = source = /note="Description of Artificial Sequence: Syntheticpolypeptide construct"
  REGION 1..128: note = source = /note="#17-PEP+"
ELVMTQTPASVSEPVGGTVTIKCQASQSISSYLAWYQQKPGQPPKLLIYAASTLASGVPSRFKGSGSGTQFTLTISDLECADAATYYCQSYYDSSSTNAFGGGTEVVVKSGGGGSGGGGSSAGILKRW

SEQ ID NO: 89 - protein, 131 aa, synthetic construct
  REGION 1..131: note = source = /note="Description of Artificial Sequence: Syntheticpolypeptide construct"
  REGION 1..131: note = source = /note="#17-PepH1"
ELVMTQTPASVSEPVGGTVTIKCQASQSISSYLAWYQQKPGQPPKLLIYAASTLASGVPSRFKGSGSGTQFTLTISDLECADAATYYCQSYYDSSSTNAFGGGTEVVVKSGGGGSGGGGSSVQQLTKRFSL

SEQ ID NO: 90 - protein, 135 aa, synthetic construct
  REGION 1..135: note = source = /note="Description of Artificial Sequence: Syntheticpolypeptide construct"
  REGION 1..135: note = source = /note="#17-PepH2"
ELVMTQTPASVSEPVGGTVTIKCQASQSISSYLAWYQQKPGQPPKLLIYAASTLASGVPSRFKGSGSGTQFTLTISDLECADAATYYCQSYYDSSSTNAFGGGTEVVVKSGGGGSGGGGSSKLFMALVAFLRFLT

SEQ ID NO: 91 - protein, 144 aa, synthetic construct
  REGION 1..144: note = source = /note="Description of Artificial Sequence: Syntheticpolypeptide construct"
  REGION 1..144: note = source = /note="#17-PepH4"
ELVMTQTPASVSEPVGGTVTIKCQASQSISSYLAWYQQKPGQPPKLLIYAASTLASGVPSRFKGSGSGTQFTLTISDLECADAATYYCQSYYDSSSTNAFGGGTEVVVKSGGGGSGGGGSSKSKAINVLRGFRKEIGRMLNILN

SEQ ID NO: 92 - protein, 131 aa, synthetic construct
  REGION 1..131: note = source = /note="Description of Artificial Sequence: Syntheticpolypeptide construct"
  REGION 1..131: note = source = /note="#19-PEP+"
ELVMTQTPSPVSAAVGGTVTISCQASQSVYNNKNLAWYQQKPGQPPKLLIYDASKLASGVSSRFKGSGSGTQFTLTISDLECDDAATYYCAGVYNSNNDACAFGGGTEVVVKSGGGGSGGGGSSAGILKRW

SEQ ID NO: 93 - protein, 134 aa, synthetic construct
  REGION 1..134: note = source = /note="Description of Artificial Sequence: Syntheticpolypeptide construct"
  REGION 1..134: note = source = /note="#19-PepH1"
ELVMTQTPSPVSAAVGGTVTISCQASQSVYNNKNLAWYQQKPGQPPKLLIYDASKLASGVSSRFKGSGSGTQFTLTISDLECDDAATYYCAGVYNSNNDACAFGGGTEVVVKSGGGGSGGGGSSVQQLTKRFSL

SEQ ID NO: 94 - protein, 138 aa, synthetic construct
  REGION 1..138: note = source = /note="Description of Artificial Sequence: Syntheticpolypeptide construct"
  REGION 1..138: note = source = /note="#19-PepH2"
ELVMTQTPSPVSAAVGGTVTISCQASQSVYNNKNLAWYQQKPGQPPKLLIYDASKLASGVSSRFKGSGSGTQFTLTISDLECDDAATYYCAGVYNSNNDACAFGGGTEVVVKSGGGGSGGGGSSKLFMALVAFLRFLT

SEQ ID NO: 95 - protein, 147 aa, synthetic construct
  REGION 1..147: note = source = /note="Description of Artificial Sequence: Syntheticpolypeptide construct"
  REGION 1..147: note = source = /note="#19-PepH4"
ELVMTQTPSPVSAAVGGTVTISCQASQSVYNNKNLAWYQQKPGQPPKLLIYDASKLASGVSSRFKGSGSGTQFTLTISDLECDDAATYYCAGVYNSNNDACAFGGGTEVVVKSGGGGSGGGGSSKSKAINVLRGFRKEIGRMLNILN

SEQ ID NO: 96 - protein, 130 aa, synthetic construct; identical to SEQ ID NO: 72
  REGION 1..130: note = source = /note="Description of Artificial Sequence: Syntheticpolypeptide construct"
  REGION 1..130: note = source = /note="#26-PEP+"

SEQ ID NO: 97 - protein, 133 aa, synthetic construct; identical to SEQ ID NO: 73
  REGION 1..133: note = source = /note="Description of Artificial Sequence: Syntheticpolypeptide construct"
  REGION 1..133: note = source = /note="#26-PepH1"

SEQ ID NO: 98 - protein, 137 aa, synthetic construct; identical to SEQ ID NO: 74
  REGION 1..137: note = source = /note="Description of Artificial Sequence: Syntheticpolypeptide construct"
  REGION 1..137: note = source = /note="#26-PepH2"

SEQ ID NO: 99 - protein, 146 aa, synthetic construct; identical to SEQ ID NO: 75
  REGION 1..146: note = source = /note="Description of Artificial Sequence: Syntheticpolypeptide construct"
  REGION 1..146: note = source = /note="#26-PepH4"

SEQ ID NO: 100 - protein, 127 aa, synthetic construct
  REGION 1..127: note = source = /note="Description of Artificial Sequence: Syntheticpolypeptide construct"
  REGION 1..127: note = source = /note="#29-PEP+"
ELDLTQTPSSVEAAVGGTVTIKCQASQSISSYLAWYQQKPGQPPKLLIYRASILASGVPSRFKASGSGTQFTLTISDLECADAATYYCQDHYGISDVAFGGGTELEILSGGGGSGGGGSSAGILKRW

SEQ ID NO: 101 - protein, 130 aa, synthetic construct
  REGION 1..130: note = source = /note="Description of Artificial Sequence: Syntheticpolypeptide construct"
  REGION 1..130: note = source = /note="#29-PepH1"
ELDLTQTPSSVEAAVGGTVTIKCQASQSISSYLAWYQQKPGQPPKLLIYRASILASGVPSRFKASGSGTQFTLTISDLECADAATYYCQDHYGISDVAFGGGTELEILSGGGGSGGGGSSVQQLTKRFSL

SEQ ID NO: 102 - protein, 134 aa, synthetic construct
  REGION 1..134: note = source = /note="Description of Artificial Sequence: Syntheticpolypeptide construct"
  REGION 1..134: note = source = /note="#29-PepH2"
ELDLTQTPSSVEAAVGGTVTIKCQASQSISSYLAWYQQKPGQPPKLLIYRASILASGVPSRFKASGSGTQFTLTISDLECADAATYYCQDHYGISDVAFGGGTELEILSGGGGSGGGGSSKLFMALVAFLRFLT

SEQ ID NO: 103 - protein, 143 aa, synthetic construct
  REGION 1..143: note = source = /note="Description of Artificial Sequence: Syntheticpolypeptide construct"
  REGION 1..143: note = source = /note="#29-PepH4"
ELDLTQTPSSVEAAVGGTVTIKCQASQSISSYLAWYQQKPGQPPKLLIYRASILASGVPSRFKASGSGTQFTLTISDLECADAATYYCQDHYGISDVAFGGGTELEILSGGGGSGGGGSSKSKAINVLRGFRKEIGRMLNILN

SEQ ID NO: 104 - protein, 131 aa, synthetic construct; identical to SEQ ID NO: 52
  REGION 1..131: note = source = /note="Description of Artificial Sequence: Syntheticpolypeptide construct"
  REGION 1..131: note = source = /note="#37-PEP+"

SEQ ID NO: 105 - protein, 134 aa, synthetic construct; identical to SEQ ID NO: 53
  REGION 1..134: note = source = /note="Description of Artificial Sequence: Syntheticpolypeptide construct"
  REGION 1..134: note = source = /note="#37-PepH1"

SEQ ID NO: 106 - protein, 138 aa, synthetic construct; identical to SEQ ID NO: 54
  REGION 1..138: note = source = /note="Description of Artificial Sequence: Syntheticpolypeptide construct"
  REGION 1..138: note = source = /note="#37-PepH2"

SEQ ID NO: 107 - protein, 147 aa, synthetic construct; identical to SEQ ID NO: 55
  REGION 1..147: note = source = /note="Description of Artificial Sequence: Syntheticpolypeptide construct"
  REGION 1..147: note = source = /note="#37-PepH4"

SEQ ID NO: 108 - protein, 129 aa, synthetic construct
  REGION 1..129: note = source = /note="Description of Artificial Sequence: Syntheticpolypeptide construct"
  REGION 1..129: note = source = /note="#53-PEP+"
ELVLTQTPASVSEPVGGTVTIKCQASQSVSDYLAWYQQKPGQPPKLLIYRASTLASGVPSRFKGSGSGTQFTLTISDLECADAATYYCQGGYAGSSYGNAFGGGTELEILSGGGGSGGGGSSAGILKRW

SEQ ID NO: 109 - protein, 132 aa, synthetic construct
  REGION 1..132: note = source = /note="Description of Artificial Sequence: Syntheticpolypeptide construct"
  REGION 1..132: note = source = /note="#53-PepH1"
ELVLTQTPASVSEPVGGTVTIKCQASQSVSDYLAWYQQKPGQPPKLLIYRASTLASGVPSRFKGSGSGTQFTLTISDLECADAATYYCQGGYAGSSYGNAFGGGTELEILSGGGGSGGGGSSVQQLTKRFSL

SEQ ID NO: 110 - protein, 136 aa, synthetic construct
  REGION 1..136: note = source = /note="Description of Artificial Sequence: Syntheticpolypeptide construct"
  REGION 1..136: note = source = /note="#53-PepH2"
ELVLTQTPASVSEPVGGTVTIKCQASQSVSDYLAWYQQKPGQPPKLLIYRASTLASGVPSRFKGSGSGTQFTLTISDLECADAATYYCQGGYAGSSYGNAFGGGTELEILSGGGGSGGGGSSKLFMALVAFLRFLT

SEQ ID NO: 111 - protein, 145 aa, synthetic construct
  REGION 1..145: note = source = /note="Description of Artificial Sequence: Syntheticpolypeptide construct"
  REGION 1..145: note = source = /note="#53-PepH4"
ELVLTQTPASVSEPVGGTVTIKCQASQSVSDYLAWYQQKPGQPPKLLIYRASTLASGVPSRFKGSGSGTQFTLTISDLECADAATYYCQGGYAGSSYGNAFGGGTELEILSGGGGSGGGGSSKSKAINVLRGFRKEIGRMLNILN

SEQ ID NO: 112 - protein, 126 aa, Lama glama
  REGION 1..126: note = source = /note="#FC5"
ASEVQLQASGGGLVQAGGSLRLSCAASGFKITHYTMGWFRQAPGKEREFVSRITWGGDNTFYSNSVKGRFTISRDNAKNTVYLQMNSLKPEDTADYYCAAGSTSTATPLRVDYWGKGTQVTVSSLE

SEQ ID NO: 113 - protein, 145 aa, synthetic construct
  REGION 1..145: note = source = /note="Description of Artificial Sequence: Syntheticpolypeptide construct"
  REGION 1..145: note = source = /note="#FC5-PEP+"
ASEVQLQASGGGLVQAGGSLRLSCAASGFKITHYTMGWFRQAPGKEREFVSRITWGGDNTFYSNSVKGRFTISRDNAKNTVYLQMNSLKPEDTADYYCAAGSTSTATPLRVDYWGKGTQVTVSSLESGGGGSGGGGSSAGILKRW

SEQ ID NO: 114 - protein, 148 aa, synthetic construct
  REGION 1..148: note = source = /note="Description of Artificial Sequence: Syntheticpolypeptide construct"
  REGION 1..148: note = source = /note="#FC5-PepH1"
ASEVQLQASGGGLVQAGGSLRLSCAASGFKITHYTMGWFRQAPGKEREFVSRITWGGDNTFYSNSVKGRFTISRDNAKNTVYLQMNSLKPEDTADYYCAAGSTSTATPLRVDYWGKGTQVTVSSLESGGGGSGGGGSSVQQLTKRFSL

SEQ ID NO: 115 - protein, 152 aa, synthetic construct
  REGION 1..152: note = source = /note="Description of Artificial Sequence: Syntheticpolypeptide construct"
  REGION 1..152: note = source = /note="#FC5-PepH2"
ASEVQLQASGGGLVQAGGSLRLSCAASGFKITHYTMGWFRQAPGKEREFVSRITWGGDNTFYSNSVKGRFTISRDNAKNTVYLQMNSLKPEDTADYYCAAGSTSTATPLRVDYWGKGTQVTVSSLESGGGGSGGGGSSKLFMALVAFLRFLT

SEQ ID NO: 116 - protein, 161 aa, synthetic construct
  REGION 1..161: note = source = /note="Description of Artificial Sequence: Syntheticpolypeptide construct"
  REGION 1..161: note = source = /note="#FC5-PepH4"
ASEVQLQASGGGLVQAGGSLRLSCAASGFKITHYTMGWFRQAPGKEREFVSRITWGGDNTFYSNSVKGRFTISRDNAKNTVYLQMNSLKPEDTADYYCAAGSTSTATPLRVDYWGKGTQVTVSSLESGGGGSGGGGSSKSKAINVLRGFRKEIGRMLNILN

SEQ ID NO: 117 - protein, 124 aa, synthetic construct
  REGION 1..124: note = source = /note="Description of Artificial Sequence: Syntheticpolypeptide"
  REGION 1..124: note = source = /note="#Abx"
DVQLVESGGGLVQPGGSLRLSCAASGFTFSNYWMYWVRQAPGKGLEWVSTISPRAAVTYYADSVKGRFTISRDNAKNTLYLQMNSLEPDDTALYYCARSLKYWHRPQSSDFASWRRGTQVTVSS

SEQ ID NO: 118 - protein, 143 aa, synthetic construct
  REGION 1..143: note = source = /note="Description of Artificial Sequence: Syntheticpolypeptide construct"
  REGION 1..143: note = source = /note="#Abx-PEP+"
DVQLVESGGGLVQPGGSLRLSCAASGFTFSNYWMYWVRQAPGKGLEWVSTISPRAAVTYYADSVKGRFTISRDNAKNTLYLQMNSLEPDDTALYYCARSLKYWHRPQSSDFASWRRGTQVTVSSSGGGGSGGGGSSAGILKRW

SEQ ID NO: 119 - protein, 146 aa, synthetic construct
  REGION 1..146: note = source = /note="Description of Artificial Sequence: Syntheticpolypeptide construct"
  REGION 1..146: note = source = /note="#Abx-PepH1"
DVQLVESGGGLVQPGGSLRLSCAASGFTFSNYWMYWVRQAPGKGLEWVSTISPRAAVTYYADSVKGRFTISRDNAKNTLYLQMNSLEPDDTALYYCARSLKYWHRPQSSDFASWRRGTQVTVSSSGGGGSGGGGSSVQQLTKRFSL

SEQ ID NO: 120 - protein, 150 aa, synthetic construct
  REGION 1..150: note = source = /note="Description of Artificial Sequence: Syntheticpolypeptide construct"
  REGION 1..150: note = source = /note="#Abx-PepH2"
DVQLVESGGGLVQPGGSLRLSCAASGFTFSNYWMYWVRQAPGKGLEWVSTISPRAAVTYYADSVKGRFTISRDNAKNTLYLQMNSLEPDDTALYYCARSLKYWHRPQSSDFASWRRGTQVTVSSSGGGGSGGGGSSKLFMALVAFLRFLT

SEQ ID NO: 121 - protein, 159 aa, synthetic construct
  REGION 1..159: note = source = /note="Description of Artificial Sequence: Syntheticpolypeptide construct"
  REGION 1..159: note = source = /note="#Abx-PepH4"
DVQLVESGGGLVQPGGSLRLSCAASGFTFSNYWMYWVRQAPGKGLEWVSTISPRAAVTYYADSVKGRFTISRDNAKNTLYLQMNSLEPDDTALYYCARSLKYWHRPQSSDFASWRRGTQVTVSSSGGGGSGGGGSSKSKAINVLRGFRKEIGRMLNILN

SEQ ID NO: 122 - protein, 119 aa, synthetic construct
  REGION 1..119: note = source = /note="Description of Artificial Sequence: Syntheticpolypeptide"
  REGION 1..119: note = source = /note="#PMP6A6"
ASAVQLVESGGGLVQPGNSLRLSCAASGFTFRSFGMSWVRQAPGKEPEWVSSISGSGSDTLYADSVKGRFTISRDNAKTTLYLQMNSLKPEDTAVYYCTIGGSLSRSSQGTQVTVSSLE

SEQ ID NO: 123 - protein, 138 aa, synthetic construct
  REGION 1..138: note = source = /note="Description of Artificial Sequence: Syntheticpolypeptide construct"
  REGION 1..138: note = source = /note="#PMP6A6-PEP+"
ASAVQLVESGGGLVQPGNSLRLSCAASGFTFRSFGMSWVRQAPGKEPEWVSSISGSGSDTLYADSVKGRFTISRDNAKTTLYLQMNSLKPEDTAVYYCTIGGSLSRSSQGTQVTVSSLESGGGGSGGGGSSAGILKRW

SEQ ID NO: 124 - protein, 141 aa, synthetic construct
  REGION 1..141: note = source = /note="Description of Artificial Sequence: Syntheticpolypeptide construct"
  REGION 1..141: note = source = /note="#PMP6A6-PepH1"
ASAVQLVESGGGLVQPGNSLRLSCAASGFTFRSFGMSWVRQAPGKEPEWVSSISGSGSDTLYADSVKGRFTISRDNAKTTLYLQMNSLKPEDTAVYYCTIGGSLSRSSQGTQVTVSSLESGGGGSGGGGSSVQQLTKRFSL

SEQ ID NO: 125 - protein, 145 aa, synthetic construct
  REGION 1..145: note = source = /note="Description of Artificial Sequence: Syntheticpolypeptide construct"
  REGION 1..145: note = source = /note="#PMP6A6-PepH2"
ASAVQLVESGGGLVQPGNSLRLSCAASGFTFRSFGMSWVRQAPGKEPEWVSSISGSGSDTLYADSVKGRFTISRDNAKTTLYLQMNSLKPEDTAVYYCTIGGSLSRSSQGTQVTVSSLESGGGGSGGGGSSKLFMALVAFLRFLT

SEQ ID NO: 126 - protein, 154 aa, synthetic construct
  REGION 1..154: note = source = /note="Description of Artificial Sequence: Syntheticpolypeptide construct"
  REGION 1..154: note = source = /note="#PMP6A6-PepH4"
ASAVQLVESGGGLVQPGNSLRLSCAASGFTFRSFGMSWVRQAPGKEPEWVSSISGSGSDTLYADSVKGRFTISRDNAKTTLYLQMNSLKPEDTAVYYCTIGGSLSRSSQGTQVTVSSLESGGGGSGGGGSSKSKAINVLRGFRKEIGRMLNILN

SEQ ID NO: 127 - protein, 100 aa, Dengue virus 2
  REGION 1..100: note = source = /note="DEN2C"
MNNQRKNARKTPFNMLKRERNRVSTVQQLTKRFSLGMLQGRGPFKLFMALVAFLRFLTIPPTAGILKRWGTIKKSKAINVLRGFRKEIGRMLNILNRRRR

SEQ ID NO: 128 - DNA, 38 bp, synthetic construct
  misc_feature 1..38: note = source = /note="Description of Artificial Sequence: Syntheticsense primer for rabbit VL domain"
  misc_feature 1..38: note = source = /note="SDV-kappa-1-F"
  source 1..38: mol_type = other DNA
gggcccaggcggccgagctcgtgmtgacccagactcca

SEQ ID NO: 129 - DNA, 38 bp, synthetic construct
  misc_feature 1..38: note = source = /note="Description of Artificial Sequence: Syntheticsense primer for rabbit VL domain"
  misc_feature 1..38: note = source = /note="SDV-kappa-2-F"
  source 1..38: mol_type = other DNA
gggcccaggcggccgagctcgatmtgacccagactcca

SEQ ID NO: 130 - DNA, 38 bp, synthetic construct
  misc_feature 1..38: note = source = /note="Description of Artificial Sequence: Syntheticsense primer for rabbit VL domain"
  misc_feature 1..38: note = source = /note="SDV-kappa-3-F"
  source 1..38: mol_type = other DNA
gggcccaggcggccgagctcgtgatgacccagactgaa

SEQ ID NO: 131 - DNA, 40 bp, synthetic construct
  misc_feature 1..40: note = source = /note="Description of Artificial Sequence: Syntheticsense primer for rabbit VL domain"
  misc_feature 1..40: note = source = /note="SDV-lambda-F"
  source 1..40: mol_type = other DNA
gggcccaggcggccgagctcgtgctgactcagtcgccctc

SEQ ID NO: 132 - DNA, 37 bp, synthetic construct
  misc_feature 1..37: note = source = /note="Description of Artificial Sequence: Syntheticantisense primer for rabbit VL domain"
  misc_feature 1..37: note = source = /note="SDV-kappa-j10-R"
  source 1..37: mol_type = other DNA
cctggccggcctggcctttgatttccacattggtgcc

SEQ ID NO: 133 - DNA, 37 bp, synthetic construct
  misc_feature 1..37: note = source = /note="Description of Artificial Sequence: Syntheticantisense primer for rabbit VL domain"
  misc_feature 1..37: note = source = /note="SDV-kappa-j0-R"
  source 1..37: mol_type = other DNA
cctggccggcctggcctaggatctccagctcggtccc

SEQ ID NO: 134 - DNA, 37 bp, synthetic construct
  misc_feature 1..37: note = source = /note="Description of Artificial Sequence: Syntheticantisense primer for rabbit VL domain"
  misc_feature 1..37: note = source = /note="SDV-kappa-j42-R"
  source 1..37: mol_type = other DNA
cctggccggcctggcctttgacsaccacctcggtccc

SEQ ID NO: 135 - DNA, 40 bp, synthetic construct
  misc_feature 1..40: note = source = /note="Description of Artificial Sequence: Syntheticantisense primer for rabbit VL domain"
  misc_feature 1..40: note = source = /note="SDV-lambda-R"
  source 1..40: mol_type = other DNA
cctggccggcctggccgcctgtgacggtcagctgggtccc